European Patent Application EP 4 613 759 A1, published September 10, 2025. Title: FRUCTOSE-1,6-DIPHOSPHATE OPTICAL PROBE, AND PREPARATION METHOD THEREFOR AND USE THEREOF. Applicant: EAST CHINA UNIVERSITY OF SCIENCE AND TECHNOLOGY. The sequence listing filed with the application follows.

SEQUENCE LISTING (23 sequences)

SEQ ID NO: 1 - protein, 340 aa, synthetic construct
MNQLIQAQKKLLPDLLVVMQKRFEILQYIRLTEPIGRRSLSASLGISERVLRGEVQFLKEQNLVEIKTNGMTLTEEGYSLLSILEDTMKDVLGLTVLEKTLKERLNLRDAIIVSGDSDQSPWVKKELGRAAVACMKKRFSGKNIVAVTGGTTIEAVAEMMTPDSKNRELLFVPARGGLGENVKNQANTICAHMAEKASGTYRLLFVPGQLSQGAYSSIIEEPSVKEVLTTIKSASMLVHGIGEAKTMAERRNTPLEDLKKIDENHAVTEAFGYYFNSDGEVVHKVHSVGMQLDDLDAIPDIIAVAGGSSKAGAIEAYFKKPRNTVLVTDEGAAKKLLRDE

SEQ ID NO: 2 - protein, 246 aa, synthetic construct
YNSDNVYIMADKQKNGIKTNFKIRHNVEDGSVQLADHYQQNTPIGDGPVLLPDNHYLSFQSVLSKDPNEKRDHMVLLEFVTAAGITLGMDELYNVDGGSGGTGSKGEELFTGVVPILVELDGDVNGHKFSVSGEGEGDATYGKLTLKLICTTGKLPVPWPTLVTTLGYGLKCFARYPDHMKQHDFFKSAMPEGYVQERTIFFKDDGNYKTRAEVKFEGDTLVNRIELKGIDFKEDGNILGHKLEYN

SEQ ID NO: 3 - protein, 242 aa, synthetic construct
VSERMYPEDGVLKSEIKKGLRLKDGGHYAAEVKTTYKAKKPVQLPGAYIVDIKLDIVSHNEDYTIVEQCERAEGRHPTGGRDELYKGGTGGSLVSKGEEDNMAIIKEFMRFKVHMEGSVNGHEFEIEGEGEGRPYEAFQTAKLKVTKGGPLPFAWDILSPQFTYGSKAYIKHPADIPDYFKLSFPEGFRWERVMNFEDGGIIHVNQDSSLQDGVFIYKVKLRGTNFPPDGPVMQKKTMGWEA

SEQ ID NO: 4 - protein, 250 aa, synthetic construct
MGGRSKKPAKNLKMPGVYYVDRRLERIKEADKETYVEQHEVAVARYCDLPSKLGHKLNGGTGGSMVSKGEELIKENMHMKLYMEGTVNNHHFKCTSEGEGKPYEGTQTMRIKVVEGGPLPFAFDILATSFMYGSKTFINHTQGIPDFFKQSFPEGFTWERVTTYEDGGVLTATQDTSLQDGCLIYNVKIRGVNFPSNGPVMQKKTLGWEASTEMLYPADGGLEGRSDMALKLVGGGHLICNLKTTYRSKK

SEQ ID NO: 5 - protein, 236 aa, synthetic construct
MVSKGEEDNMAIIKEFMRFKVHMEGSVNGHEFEIEGEGEGRPYEGTQTAKLKVTKGGPLPFAWDILSPQFMYGSKAYVKHPADIPDYLKLSFPEGFKWERVMNFEDGGVVTVTQDSSLQDGEFIYKVKLRGTNFPSDGPVMQKKTMGWEASSERMYPEDGALKGEIKQRLKLKDGGHYDAEVKTTYKAKKPVQLPGAYNVNIKLDITSHNEDYTIVEQYERAEGRHSTGGMDELYK

SEQ ID NO: 6 - protein, 241 aa, synthetic construct
NVYIKADKQKNGIKANFKIRHNIEDGGVQLAYHYQQNTPIGDGPVLLPDNHYLSVQSILSKDPNEKRDHMVLLEFVTAAGITLGMDELYKGGTGGSMVSKGEELFTGVVPIQVELDGDVNGHKFSVSGEGEGDATYGKLTLKFICTTGKLPVPWPTLVTTLTYGVQCFSRYPDHMKQHDFFKSAMPEGYIQERTIFFKDDGNYKTRAEVKFEGDTLVNRIELKGIDFKEDGNILGHKLEYN

SEQ ID NO: 7 - protein, 243 aa, synthetic construct
NVYIKADKQKNGIKANFKIRHNIEGGGVQLAYHYQQNTPIGDGPVLLPDNHYLSVQSILSKDPNEKRDHMVLLEFVTAAGITLGMDELYKGGTGGSESMVSKGEELFTGVVPIQVELDGDVNGHKFSVSGEGEGDATYGKLTLKFICTTGKLPVPWPTLVTTLSHGVQCFSRYPDHMKQHDFFKSAMPGGYIQERTIFFKDDGNYKTRAEVKFEGDTLVNRIELKGIDFKEDGNILGHKLEYN

SEQ ID NO: 8 - protein, 233 aa, synthetic construct
MSELITENMHMKLYMEGTVNNHHFKCTSEGEGKPYEGTQTMRIKVVEGGPLPFAFDILATSFMYGSKTFINHTQGIPDFFKQSFPEGFTWERVTTYEDGGVLTATQDTSLQDGCLIYNVKIRGVNFPSNGPVMQKKTLGWEASTEMLYPADGGLEGRADMALKLVGGGHLICNLKTTYRSKKPAKNLKMPGVYYVDRRLERIKEADKETYVEQHEVAVARYCDLPSKLGHKLN

SEQ ID NO: 9 - protein, 242 aa, synthetic construct
VSERMYPEDGALKSEIKKGLRLKDGGHYAAEVKTTYKAKKPVQLPGAYIVDIKLDIVSHNEDYTIVEQCERAEGRHSTGGMDELYKGGTGGSLVSKGEEDNMAIIKEFMRFKVHMEGSVNGHEFEIEGEGEGRPYEAFQTAKLKVTKGGPLPFAWDILSPQFMYGSKAYIKHPADIPDYFKLSFPEGFRWERVMNFEDGGIIHVNQDSSLQDGVFIYKVKLRGTNFPPDGPVMQKKTMGWEA

SEQ ID NO: 10 - protein, 501 aa, synthetic construct
SNAKDVLGLTLLEKTLKERLNLKDAIIVSGDSDQSPWVKKEMGRAAVACMKKRFSGKNIVAVTGGTTIEAVAEMMTPDSKNRELLFVPARGYNSDNVYIMADKQKNGIKTNFKIRHNVEDGSVQLADHYQQNTPIGDGPVLLPDNHYLSFQSVLSKDPNEKRDHMVLLEFVTAAGITLGMDELYNVDGGSGGTGSKGEELFTGVVPILVELDGDVNGHKFSVSGEGEGDATYGKLTLKLICTTGKLPVPWPTLVTTLGYGLKCFARYPDHMKQHDFFKSAMPEGYVQERTIFFKDDGNYKTRAEVKFEGDTLVNRIELKGIDFKEDGNILGHKLEYNMNGEDVKNQANTICAHMAEKASGTYRLLFVPGQLSQGAYSSIIEEPSVKEVLNTIKSASMLVHGIGEAKTMAQRRNTPLEDLKKIDDNDAVTEAFGYYFNADGEVVHKVHSVGMQLDDIDAIPDIIAVAGGSSKAEAIEAYFKKPRNTVLVTDEGAAKKLLRDE

SEQ ID NO: 11 - protein, 501 aa, synthetic construct
SNAKDVLGLTLLEKTLKERLNLKDAIIVSGDSDQSPWVKKEMGRAAVACMKKRFSGKNIVAVTGGTTIEAVAEMMTPDSKNRELLFVPARGYNSDNVYIMADKQKNGIKTNFKIRHNVEDGSVQLADHYQQNTPIGDGPVLLPDNHYLSFQSVLSKDPNEKRDHMVLLEFVTAAGITLGMDELYNVDGGSGGTGSKGEELFTGVVPILVELDGDVNGHKFSVSGEGEGDATYGKLTLKLICTTGKLPVPWPTLVTTLGYGLKCFARYPDHMKQHDFFKSAMPEGYVQERTIFFKDDGNYKTRAEVKFEGDTLVNRIELKGIDFKEDGNILGHKLEYNMNGEDVKNAANTICAHMAEKASGTYRLLFVPGQLSQGAYSSIIEEPSVKEVLNTIKSASMLVHGIGEAKTMAQRRNTPLEDLKKIDDNDAVTEAFGYYFNADGEVVHKVHSVGMQLDDIDAIPDIIAVAGGSSKAEAIEAYFKKPRNTVLVTDEGAAKKLLRDE

SEQ ID NO: 12 - protein, 501 aa, synthetic construct
SNAKDVLGLTLLEKTLKERLNLKDAIIVSGDSDQSPWVKKEMGRAAVACMKKRFSGKNIVAVTGGTTIEAVAEMMTPDSKNRELLFVPARGYNSDNVYIMADKQKNGIKTNFKIRHNVEDGSVQLADHYQQNTPIGDGPVLLPDNHYLSFQSVLSKDPNEKRDHMVLLEFVTAAGITLGMDELYNVDGGSGGTGSKGEELFTGVVPILVELDGDVNGHKFSVSGEGEGDATYGKLTLKLICTTGKLPVPWPTLVTTLGYGLKCFARYPDHMKQHDFFKSAMPEGYVQERTIFFKDDGNYKTRAEVKFEGDTLVNRIELKGIDFKEDGNILGHKLEYNMNGEDVKNTANTICAHMAEKASGTYRLLFVPGQLSQGAYSSIIEEPSVKEVLNTIKSASMLVHGIGEAKTMAQRRNTPLEDLKKIDDNDAVTEAFGYYFNADGEVVHKVHSVGMQLDDIDAIPDIIAVAGGSSKAEAIEAYFKKPRNTVLVTDEGAAKKLLRDE

SEQ ID NO: 13 - protein, 501 aa, synthetic construct
SNAKDVLGLTLLEKTLKERLNLKDAIIVSGDSDQSPWVKKEMGRAAVACMKKRFSGKNIVAVTGGTTIEAVAEMMTPDSKNRELLFVPARGYNSDNVYIMADKQKNGIKTNFKIRHNVEDGSVQLADHYQQNTPIGDGPVLLPDNHYLSFQSVLSKDPNEKRDHMVLLEFVTAAGITLGMDELYNVDGGSGGTGSKGEELFTGVVPILVELDGDVNGHKFSVSGEGEGDATYGKLTLKLICTTGKLPVPWPTLVTTLGYGLKCFARYPDHMKQHDFFKSAMPEGYVQERTIFFKDDGNYKTRAEVKFEGDTLVNRIELKGIDFKEDGNILGHKLEYNMNGEDVKNDANTICAHMAEKASGTYRLLFVPGQLSQGAYSSIIEEPSVKEVLNTIKSASMLVHGIGEAKTMAQRRNTPLEDLKKIDDNDAVTEAFGYYFNADGEVVHKVHSVGMQLDDIDAIPDIIAVAGGSSKAEAIEAYFKKPRNTVLVTDEGAAKKLLRDE

SEQ ID NO: 14 - protein, 500 aa, synthetic construct
SNAKDVLGLTLLEKTLKERLNLKDAIIVSGDSDQSPWVKKEMGRAAVACMKKRFSGKNIVAVTGGTTIEAVAEMMTPDSKNRELLFVPARGLLGEEGVNSDNVYIMADKQKNGIKTNFKIRHNVEDGSVQLADHYQQNTPIGDGPVLLPDNHYLSFQSVLSKDPNEKRDHMVLLEFVTAAGITLGMDELYNVDGGSGGTGSKGEELFTGVVPILVELDGDVNGHKFSVSGEGEGDATYGKLTLKLICTTGKLPVPWPTLVTTLGYGLKCFARYPDHMKQHDFFKSAMPEGYVQERTIFFKDDGNYKTRAEVKFEGDTLVNRIELKGIDFKEDGNILGHKLEYNVPANTICAHMAEKASGTYRLLFVPGQLSQGAYSSIIEEPSVKEVLNTIKSASMLVHGIGEAKTMAQRRNTPLEDLKKIDDNDAVTEAFGYYFNADGEVVHKVHSVGMQLDDIDAIPDIIAVAGGSSKAEAIEAYFKKPRNTVLVTDEGAAKKLLRDE

SEQ ID NO: 15 - protein, 500 aa, synthetic construct
SNAKDVLGLTLLEKTLKERLNLKDAIIVSGDSDQSPWVKKEMGRAAVACMKKRFSGKNIVAVTGGTTIEAVAEMMTPDSKNRELLFVPARGLLGEEGINSDNVYIMADKQKNGIKTNFKIRHNVEDGSVQLADHYQQNTPIGDGPVLLPDNHYLSFQSVLSKDPNEKRDHMVLLEFVTAAGITLGMDELYNVDGGSGGTGSKGEELFTGVVPILVELDGDVNGHKFSVSGEGEGDATYGKLTLKLICTTGKLPVPWPTLVTTLGYGLKCFARYPDHMKQHDFFKSAMPEGYVQERTIFFKDDGNYKTRAEVKFEGDTLVNRIELKGIDFKEDGNILGHKLEYNVPANTICAHMAEKASGTYRLLFVPGQLSQGAYSSIIEEPSVKEVLNTIKSASMLVHGIGEAKTMAQRRNTPLEDLKKIDDNDAVTEAFGYYFNADGEVVHKVHSVGMQLDDIDAIPDIIAVAGGSSKAEAIEAYFKKPRNTVLVTDEGAAKKLLRDE

SEQ ID NO: 16 - protein, 500 aa, synthetic construct
SNAKDVLGLTLLEKTLKERLNLKDAIIVSGDSDQSPWVKKEMGRAAVACMKKRFSGKNIVAVTGGTTIEAVAEMMTPDSKNRELLFVPARGGLGEEGVNSDNVYIMADKQKNGIKTNFKIRHNVEDGSVQLADHYQQNTPIGDGPVLLPDNHYLSFQSVLSKDPNEKRDHMVLLEFVTAAGITLGMDELYNVDGGSGGTGSKGEELFTGVVPILVELDGDVNGHKFSVSGEGEGDATYGKLTLKLICTTGKLPVPWPTLVTTLGYGLKCFARYPDHMKQHDFFKSAMPEGYVQERTIFFKDDGNYKTRAEVKFEGDTLVNRIELKGIDFKEDGNILGHKLEYNVPANTICAHMAEKASGTYRLLFVPGQLSQGAYSSIIEEPSVKEVLNTIKSASMLVHGIGEAKTMAQRRNTPLEDLKKIDDNDAVTEAFGYYFNADGEVVHKVHSVGMQLDDIDAIPDIIAVAGGSSKAEAIEAYFKKPRNTVLVTDEGAAKKLLRDE

SEQ ID NO: 17 - DNA, 1503 bp, synthetic construct
  source 1..1503: mol_type = other DNA
tctaatgctaaagatgttctgggcctgaccctgctggagaagaccctgaaagaacgtctgaacctgaaagatgctatcattgtgagcggcgacagcgatcagagcccgtgggtgaagaaagagatgggtcgtgccgcggtggcgtgcatgaagaaacgcttcagcggcaagaacatcgtggctgtgaccggcggtaccaccattgaggcggtggctgaaatgatgaccccggacagcaaaaaccgtgagctgctgtttgtgccagctcgcggctacaacagcgacaacgtctatatcatggccgacaagcagaagaacggcatcaaggccaacttcaagatccgccacaacgtcgaggacggcagcgtgcagctcgccgaccactaccagcagaacacccccatcggcgacggccccgtgctgctgcccgacaaccactacctgagcttccagtccgtcctgagcaaagaccccaacgagaagcgcgatcacatggtcctgctggagttcgtgaccgccgccgggatcactctcggcatggacgagctgtacaacgtggatggcggtagcggtggcaccggcagcaagggcgaggagctgttcaccggggtggtgcccatcctggtcgagctggacggcgacgtaaacggccacaagttcagcgtgtccggcgagggcgagggcgatgccacctacggcaagctgaccctgaagctgatctgcaccaccggcaagctgcccgtgccctggcccaccctcgtgaccaccctcggctacggcctgaagtgcttcgcccgctaccccgaccacatgaagcagcacgacttcttcaagtccgccatgcccgaaggctacgtccaggagcgcaccatcttcttcaaggacgacggcaactacaagacccgcgccgaggtgaagttcgagggcgacaccctggtgaaccgcatcgagctgaagggcatcggcttcaaggaggacggcaacatcctggggcacaagctggagtacaacatgaatggtgaagatgtgaagaaccaggccaacaccatctgcgcgcacatggctgagaaagccagcggtacctatcgcctgctgtttgtgccgggtcagctgagccagggtgcttatagcagcatcattgaggaaccgagcgtgaaggaagtgctgaacaccatcaaaagcgccagcatgctggtgcacggcattggcgaggcgaagaccatggctcagcgtcgcaacaccccgctggaagacctgaagaaaatcgacgataacgatgccgtgaccgaggccttcggctactacttcaacgcggacggtgaagtggtgcacaaggtgcacagcgtgggtatgcagctggacgatatcgacgccattccggatatcattgccgtggcgggcggtagcagcaaagctgaggccattgaagcgtactttaagaaaccgcgtaataccgtgctggtgaccgatgagggtgctgccaagaaactgctgcgcgatgaa

SEQ ID NO: 18 - DNA, 1503 bp, synthetic construct
  source 1..1503: mol_type = other DNA
tctaatgctaaagatgttctgggcctgaccctgctggagaagaccctgaaagaacgtctgaacctgaaagatgctatcattgtgagcggcgacagcgatcagagcccgtgggtgaagaaagagatgggtcgtgccgcggtggcgtgcatgaagaaacgcttcagcggcaagaacatcgtggctgtgaccggcggtaccaccattgaggcggtggctgaaatgatgaccccggacagcaaaaaccgtgagctgctgtttgtgccagctcgcggctacaacagcgacaacgtctatatcatggccgacaagcagaagaacggcatcaaggccaacttcaagatccgccacaacgtcgaggacggcagcgtgcagctcgccgaccactaccagcagaacacccccatcggcgacggccccgtgctgctgcccgacaaccactacctgagcttccagtccgtcctgagcaaagaccccaacgagaagcgcgatcacatggtcctgctggagttcgtgaccgccgccgggatcactctcggcatggacgagctgtacaacgtggatggcggtagcggtggcaccggcagcaagggcgaggagctgttcaccggggtggtgcccatcctggtcgagctggacggcgacgtaaacggccacaagttcagcgtgtccggcgagggcgagggcgatgccacctacggcaagctgaccctgaagctgatctgcaccaccggcaagctgcccgtgccctggcccaccctcgtgaccaccctcggctacggcctgaagtgcttcgcccgctaccccgaccacatgaagcagcacgacttcttcaagtccgccatgcccgaaggctacgtccaggagcgcaccatcttcttcaaggacgacggcaactacaagacccgcgccgaggtgaagttcgagggcgacaccctggtgaaccgcatcgagctgaagggcatcggcttcaaggaggacggcaacatcctggggcacaagctggagtacaacatgaatggtgaagatgtgaagaacgccgccaacaccatctgcgcgcacatggctgagaaagccagcggtacctatcgcctgctgtttgtgccgggtcagctgagccagggtgcttatagcagcatcattgaggaaccgagcgtgaaggaagtgctgaacaccatcaaaagcgccagcatgctggtgcacggcattggcgaggcgaagaccatggctcagcgtcgcaacaccccgctggaagacctgaagaaaatcgacgataacgatgccgtgaccgaggccttcggctactacttcaacgcggacggtgaagtggtgcacaaggtgcacagcgtgggtatgcagctggacgatatcgacgccattccggatatcattgccgtggcgggcggtagcagcaaagctgaggccattgaagcgtactttaagaaaccgcgtaataccgtgctggtgaccgatgagggtgctgccaagaaactgctgcgcgatgaa

SEQ ID NO: 19 - DNA, 1503 bp, synthetic construct
  source 1..1503: mol_type = other DNA
tctaatgctaaagatgttctgggcctgaccctgctggagaagaccctgaaagaacgtctgaacctgaaagatgctatcattgtgagcggcgacagcgatcagagcccgtgggtgaagaaagagatgggtcgtgccgcggtggcgtgcatgaagaaacgcttcagcggcaagaacatcgtggctgtgaccggcggtaccaccattgaggcggtggctgaaatgatgaccccggacagcaaaaaccgtgagctgctgtttgtgccagctcgcggctacaacagcgacaacgtctatatcatggccgacaagcagaagaacggcatcaaggccaacttcaagatccgccacaacgtcgaggacggcagcgtgcagctcgccgaccactaccagcagaacacccccatcggcgacggccccgtgctgctgcccgacaaccactacctgagcttccagtccgtcctgagcaaagaccccaacgagaagcgcgatcacatggtcctgctggagttcgtgaccgccgccgggatcactctcggcatggacgagctgtacaacgtggatggcggtagcggtggcaccggcagcaagggcgaggagctgttcaccggggtggtgcccatcctggtcgagctggacggcgacgtaaacggccacaagttcagcgtgtccggcgagggcgagggcgatgccacctacggcaagctgaccctgaagctgatctgcaccaccggcaagctgcccgtgccctggcccaccctcgtgaccaccctcggctacggcctgaagtgcttcgcccgctaccccgaccacatgaagcagcacgacttcttcaagtccgccatgcccgaaggctacgtccaggagcgcaccatcttcttcaaggacgacggcaactacaagacccgcgccgaggtgaagttcgagggcgacaccctggtgaaccgcatcgagctgaagggcatcggcttcaaggaggacggcaacatcctggggcacaagctggagtacaacatgaatggtgaagatgtgaagaacaccgccaacaccatctgcgcgcacatggctgagaaagccagcggtacctatcgcctgctgtttgtgccgggtcagctgagccagggtgcttatagcagcatcattgaggaaccgagcgtgaaggaagtgctgaacaccatcaaaagcgccagcatgctggtgcacggcattggcgaggcgaagaccatggctcagcgtcgcaacaccccgctggaagacctgaagaaaatcgacgataacgatgccgtgaccgaggccttcggctactacttcaacgcggacggtgaagtggtgcacaaggtgcacagcgtgggtatgcagctggacgatatcgacgccattccggatatcattgccgtggcgggcggtagcagcaaagctgaggccattgaagcgtactttaagaaaccgcgtaataccgtgctggtgaccgatgagggtgctgccaagaaactgctgcgcgatgaa

SEQ ID NO: 20 - DNA, 1503 bp, synthetic construct
  source 1..1503: mol_type = other DNA
tctaatgctaaagatgttctgggcctgaccctgctggagaagaccctgaaagaacgtctgaacctgaaagatgctatcattgtgagcggcgacagcgatcagagcccgtgggtgaagaaagagatgggtcgtgccgcggtggcgtgcatgaagaaacgcttcagcggcaagaacatcgtggctgtgaccggcggtaccaccattgaggcggtggctgaaatgatgaccccggacagcaaaaaccgtgagctgctgtttgtgccagctcgcggctacaacagcgacaacgtctatatcatggccgacaagcagaagaacggcatcaaggccaacttcaagatccgccacaacgtcgaggacggcagcgtgcagctcgccgaccactaccagcagaacacccccatcggcgacggccccgtgctgctgcccgacaaccactacctgagcttccagtccgtcctgagcaaagaccccaacgagaagcgcgatcacatggtcctgctggagttcgtgaccgccgccgggatcactctcggcatggacgagctgtacaacgtggatggcggtagcggtggcaccggcagcaagggcgaggagctgttcaccggggtggtgcccatcctggtcgagctggacggcgacgtaaacggccacaagttcagcgtgtccggcgagggcgagggcgatgccacctacggcaagctgaccctgaagctgatctgcaccaccggcaagctgcccgtgccctggcccaccctcgtgaccaccctcggctacggcctgaagtgcttcgcccgctaccccgaccacatgaagcagcacgacttcttcaagtccgccatgcccgaaggctacgtccaggagcgcaccatcttcttcaaggacgacggcaactacaagacccgcgccgaggtgaagttcgagggcgacaccctggtgaaccgcatcgagctgaagggcatcggcttcaaggaggacggcaacatcctggggcacaagctggagtacaacatgaatggtgaagatgtgaagaacgatgccaacaccatctgcgcgcacatggctgagaaagccagcggtacctatcgcctgctgtttgtgccgggtcagctgagccagggtgcttatagcagcatcattgaggaaccgagcgtgaaggaagtgctgaacaccatcaaaagcgccagcatgctggtgcacggcattggcgaggcgaagaccatggctcagcgtcgcaacaccccgctggaagacctgaagaaaatcgacgataacgatgccgtgaccgaggccttcggctactacttcaacgcggacggtgaagtggtgcacaaggtgcacagcgtgggtatgcagctggacgatatcgacgccattccggatatcattgccgtggcgggcggtagcagcaaagctgaggccattgaagcgtactttaagaaaccgcgtaataccgtgctggtgaccgatgagggtgctgccaagaaactgctgcgcgatgaa

SEQ ID NO: 21 - DNA, 1500 bp, synthetic construct
  source 1..1500: mol_type = other DNA
tctaatgctaaagatgttctgggcctgaccctgctggagaagaccctgaaagaacgtctgaacctgaaagatgctatcattgtgagcggcgacagcgatcagagcccgtgggtgaagaaagagatgggtcgtgccgcggtggcgtgcatgaagaaacgcttcagcggcaagaacatcgtggctgtgaccggcggtaccaccattgaggcggtggctgaaatgatgaccccggacagcaaaaaccgtgagctgctgtttgtgccagctcgcggcttgcttggtgaagaaggcgtaaacagcgacaacgtctatatcatggccgacaagcagaagaacggcatcaagaccaacttcaagatccgccacaacgtcgaggacggcagcgtgcagctcgccgaccactaccagcagaacacccccatcggcgacggccccgtgctgctgcccgacaaccactacctgagcttccagtccgtcctgagcaaagaccccaacgagaagcgcgatcacatggtcctgctggagttcgtgaccgccgccgggatcactctcggcatggacgagctgtacaacgtggatggcggtagcggtggcaccggcagcaagggcgaggagctgttcaccggggtggtgcccatcctggtcgagctggacggcgacgtaaacggccacaagttcagcgtgtccggcgagggcgagggcgatgccacctacggcaagctgaccctgaagctgatctgcaccaccggcaagctgcccgtgccctggcccaccctcgtgaccaccctcggctacggcctgaagtgcttcgcccgctaccccgaccacatgaagcagcacgacttcttcaagtccgccatgcccgaaggctacgtccaggagcgcaccatcttcttcaaggacgacggcaactacaagacccgcgccgaggtgaagttcgagggcgacaccctggtgaaccgcatcgagctgaagggcatcgacttcaaggaggacggcaacatcctggggcacaagctggagtacaacgtgccggccaacaccatctgcgcgcacatggctgagaaagccagcggtacctatcgcctgctgtttgtgccgggtcagctgagccagggtgcttatagcagcatcattgaggaaccgagcgtgaaggaagtgctgaacaccatcaaaagcgccagcatgctggtgcacggcattggcgaggcgaagaccatggctcagcgtcgcaacaccccgctggaagacctgaagaaaatcgacgataacgatgccgtgaccgaggccttcggctactacttcaacgcggacggtgaagtggtgcacaaggtgcacagcgtgggtatgcagctggacgatatcgacgccattccggatatcattgccgtggcgggcggtagcagcaaagctgaggccattgaagcgtactttaagaaaccgcgtaataccgtgctggtgaccgatgagggtgctgccaagaaactgctgcgcgatgaa

SEQ ID NO: 22 - DNA, 1500 bp, synthetic construct
  source 1..1500: mol_type = other DNA
tctaatgctaaagatgttctgggcctgaccctgctggagaagaccctgaaagaacgtctgaacctgaaagatgctatcattgtgagcggcgacagcgatcagagcccgtgggtgaagaaagagatgggtcgtgccgcggtggcgtgcatgaagaaacgcttcagcggcaagaacatcgtggctgtgaccggcggtaccaccattgaggcggtggctgaaatgatgaccccggacagcaaaaaccgtgagctgctgtttgtgccagctcgcggcttgcttggtgaagaaggcatcaacagcgacaacgtctatatcatggccgacaagcagaagaacggcatcaagaccaacttcaagatccgccacaacgtcgaggacggcagcgtgcagctcgccgaccactaccagcagaacacccccatcggcgacggccccgtgctgctgcccgacaaccactacctgagcttccagtccgtcctgagcaaagaccccaacgagaagcgcgatcacatggtcctgctggagttcgtgaccgccgccgggatcactctcggcatggacgagctgtacaacgtggatggcggtagcggtggcaccggcagcaagggcgaggagctgttcaccggggtggtgcccatcctggtcgagctggacggcgacgtaaacggccacaagttcagcgtgtccggcgagggcgagggcgatgccacctacggcaagctgaccctgaagctgatctgcaccaccggcaagctgcccgtgccctggcccaccctcgtgaccaccctcggctacggcctgaagtgcttcgcccgctaccccgaccacatgaagcagcacgacttcttcaagtccgccatgcccgaaggctacgtccaggagcgcaccatcttcttcaaggacgacggcaactacaagacccgcgccgaggtgaagttcgagggcgacaccctggtgaaccgcatcgagctgaagggcatcgacttcaaggaggacggcaacatcctggggcacaagctggagtacaacgtgccggccaacaccatctgcgcgcacatggctgagaaagccagcggtacctatcgcctgctgtttgtgccgggtcagctgagccagggtgcttatagcagcatcattgaggaaccgagcgtgaaggaagtgctgaacaccatcaaaagcgccagcatgctggtgcacggcattggcgaggcgaagaccatggctcagcgtcgcaacaccccgctggaagacctgaagaaaatcgacgataacgatgccgtgaccgaggccttcggctactacttcaacgcggacggtgaagtggtgcacaaggtgcacagcgtgggtatgcagctggacgatatcgacgccattccggatatcattgccgtggcgggcggtagcagcaaagctgaggccattgaagcgtactttaagaaaccgcgtaataccgtgctggtgaccgatgagggtgctgccaagaaactgctgcgcgatgaa

SEQ ID NO: 23 - DNA, 1500 bp, synthetic construct
  source 1..1500: mol_type = other DNA
tctaatgctaaagatgttctgggcctgaccctgctggagaagaccctgaaagaacgtctgaacctgaaagatgctatcattgtgagcggcgacagcgatcagagcccgtgggtgaagaaagagatgggtcgtgccgcggtggcgtgcatgaagaaacgcttcagcggcaagaacatcgtggctgtgaccggcggtaccaccattgaggcggtggctgaaatgatgaccccggacagcaaaaaccgtgagctgctgtttgtgccagctcgcggcggtcttggtgaagaaggcgtaaacagcgacaacgtctatatcatggccgacaagcagaagaacggcatcaagaccaacttcaagatccgccacaacgtcgaggacggcagcgtgcagctcgccgaccactaccagcagaacacccccatcggcgacggccccgtgctgctgcccgacaaccactacctgagcttccagtccgtcctgagcaaagaccccaacgagaagcgcgatcacatggtcctgctggagttcgtgaccgccgccgggatcactctcggcatggacgagctgtacaacgtggatggcggtagcggtggcaccggcagcaagggcgaggagctgttcaccggggtggtgcccatcctggtcgagctggacggcgacgtaaacggccacaagttcagcgtgtccggcgagggcgagggcgatgccacctacggcaagctgaccctgaagctgatctgcaccaccggcaagctgcccgtgccctggcccaccctcgtgaccaccctcggctacggcctgaagtgcttcgcccgctaccccgaccacatgaagcagcacgacttcttcaagtccgccatgcccgaaggctacgtccaggagcgcaccatcttcttcaaggacgacggcaactacaagacccgcgccgaggtgaagttcgagggcgacaccctggtgaaccgcatcgagctgaagggcatcgacttcaaggaggacggcaacatcctggggcacaagctggagtacaacgtgccggccaacaccatctgcgcgcacatggctgagaaagccagcggtacctatcgcctgctgtttgtgccgggtcagctgagccagggtgcttatagcagcatcattgaggaaccgagcgtgaaggaagtgctgaacaccatcaaaagcgccagcatgctggtgcacggcattggcgaggcgaagaccatggctcagcgtcgcaacaccccgctggaagacctgaagaaaatcgacgataacgatgccgtgaccgaggccttcggctactacttcaacgcggacggtgaagtggtgcacaaggtgcacagcgtgggtatgcagctggacgatatcgacgccattccggatatcattgccgtggcgggcggtagcagcaaagctgaggccattgaagcgtactttaagaaaccgcgtaataccgtgctggtgaccgatgagggtgctgccaagaaactgctgcgcgatgaa